European Patent Application EP 4 269 604 A2, published November 1, 2023. Title: BIOELECTRONIC CIRCUITS, SYSTEMS AND METHODS FOR PREPARING AND USING THEM. Applicant: ARIZONA BOARD OF REGENTS ON BEHALF OF ARIZONA STATE UNIVERSITY. Application EP. The sequence listing filed with the application follows.

SEQUENCE LISTING (7 sequences)

SEQ ID NO: 1 - protein, 12 aa, synthetic construct
CALDRWEKIRLR

SEQ ID NO: 2 - protein, 17 aa, synthetic construct
CHNTPVYKLDISEATQV

SEQ ID NO: 3 - protein, 12 aa, synthetic construct
GNSTNGTSNGSS

SEQ ID NO: 4 - protein, 15 aa, synthetic construct
GLNDIFEAQKIEWHE

SEQ ID NO: 5 - protein, 38 aa, synthetic construct
MGSSHHHHHHSSGLVPRGSGLNDIFEAQKIEWHEGASS

SEQ ID NO: 6 - protein, 12 aa, synthetic construct
GGSGGSGGSGGS

SEQ ID NO: 7 - protein, 12 aa, synthetic construct
GDSTDGTSDGSS